European Patent Application EP 4 331 603 A1, published March 6, 2024. Title: ANTI-MASP2 ANTIBODY, ANTIGEN-BINDING FRAGMENT THEREOF AND MEDICAL USE THEREOF. Applicant: JIANGSU HENGRUI PHARMACEUTICALS CO., LTD. SHANGHAI SHENGDI PHARMACEUTICAL CO., LTD. The sequence listing filed with the application follows.

SEQUENCE LISTING (61 sequences)

SEQ ID NO: 1 - protein, 707 aa, Artificial sequence
  Human MASP2A protein
MEFGLSWLFLVAILKGVQCTPLGPKWPEPVFGRLASPGFPGEYANDQERRWTLTAPPGYRLRLYFTHFDLELSHLCEYDFVKLSSGAKVLATLCGQESTDTERAPGKDTFYSLGSSLDITFRSDYSNEKPFTGFEAFYAAEDIDECQVAPGEAPTCDHHCHNHLGGFYCSCRAGYVLHRNKRTCSALCSGQVFTQRSGELSSPEYPRPYPKLSSCTYSISLEEGFSVILDFVESFDVETHPETLCPYDFLKIQTDREEHGPFCGKTLPHRIETKSNTVTITFVTDESGDHTGWKIHYTSTAQPCPYPMAPPNGHVSPVQAKYILKDSFSIFCETGYELLQGHLPLKSFTAVCQKDGSWDRPMPACSIVDCGPPDDLPSGRVEYITGPGVTTYKAVIQYSCEETFYTMKVNDGKYVCEADGFWTSSKGEKSLPVCEPVCGLSARTTGGRIYGGQKAKPGDFPWQVLILGGTTAAGALLYDNWVLTAAHAVYEQKHDASALDIRMGTLKRLSPHYTQAWSEAVFIHEGYTHDAGFDNDIALIKLNNKVVINSNITPICLPRKEAESFMRTDDIGTASGWGLTQRGFLARNLMYVDIPIVDHQKCTAAYEKPPYPRGSVTANMLCAGLESGGKDSCRGDAGGALVFLDSETERWFVGGIVSWGSMNCGEAGQYGVYTKVINYIPWIENIISDFGGSDYKDDDDKHHHHHH

SEQ ID NO: 2 - protein, 707 aa, Artificial sequence
  Monkey MASP2A protein
MEFGLSWLFLVAILKGVQCTPLGPKWPEPVFGRLASPGFPGEYANDQERRWTLTAPPGYRLRLYFTHFDLELSHLCEYDFVKLSSGAKVLATLCGHESTDTERAPGNDTFYSLGSSLDITFRSDYSNEKPFTGFEAFYAAEDIDECQVAPGEAPACDHHCHNHLGGFYCSCRVGYILHRNKRTCSALCSGQVFTQRSGELSSPEYPQPYPKLSSCTYSIRLEEGFSVILDFVESFDVETHPETLCPYDFLKIQIDSEEHGPFCGKTLPRRIETKSNTVTITFVTDESGDHTGWKIHYTSTAQPCPYPMAPPNGHLSPVQAKYILKDSFSIFCEPGYELLQGHLPLKSFAAVCQKDGSWDQPMPSCSIVDCGPPDDLPSGRVEYITGPEVTTYKAVIQYSCEETFYTMKVNDGKYVCEADGFWTSSKGERSPPVCEPVCGLSARTTGGRIYGGQKAKPGDFPWQVLILGGSTAAGALLYDNWVLTAAHAIYEQKHDASSLDIRLGALKRLSPHYTQAWAEAVFIHEGYTHDAGFDNDIALIKLNNKVVINSNITPICLPRKEAESFMRTDDIGTASGWGLTQRGLLARNLMYVDIPIVDHQKCTAAYEKPPYSGGSVTANMLCAGLESGGKDSCRGDAGGALVFLDNETQRWFVGGIVSWGSMNCGEAGQYGVYTKVINYIPWIKNIISNFGGSDYKDDDDKHHHHHH

SEQ ID NO: 3 - protein, 706 aa, Artificial sequence
  Murine MASP2A protein
MEFGLSWLFLVAILKGVQCTPLGSKWPEPVFGRLVSPGFPEKYADHQDRSWTLTAPPGYRLRLYFTHFDLELSYRCEYDFVKLSSGTKVLATLCGQESTDTEQAPGNDTFYSLGPSLKVTFHSDYSNEKPFTGFEAFYAAEDVDECRVSLGDSVPCDHYCHNYLGGYYCSCRAGYVLHQNKHTCSALCSGQVFTGRSGYLSSPEYPQPYPKLSSCTYSIRLEDGFSVILDFVESFDVETHPEAQCPYDSLKIQTDKGEHGPFCGKTLPPRIETDSHKVTITFATDESGNHTGWKIHYTSTARPCPDPTAPPNGSISPVQAIYVLKDRFSVFCKTGFELLQGSVPLKSFTAVCQKDGSWDRPMPECSIIDCGPPDDLPNGHVDYITGPEVTTYKAVIQYSCEETFYTMSSNGKYVCEADGFWTSSKGEKLPPVCEPVCGLSTHTIGGRIVGGQPAKPGDFPWQVLLLGQTTAAAGALIHDNWVLTAAHAVYEKRMAASSLNIRMGILKRLSPHYTQAWPEEIFIHEGYTHGAGFDNDIALIKLKNKVTINGSIMPVCLPRKEAASLMRTDFTGTVAGWGLTQKGLLARNLMFVDIPIADHQKCTAVYEKLYPGVRVSANMLCAGLETGGKDSCRGDAGGALVFLDNETQRWFVGGIVSWGSINCGAADQYGVYTKVINYIPWIENIISNFGGSDYKDDDDKHHHHHH

SEQ ID NO: 4 - protein, 421 aa, Artificial sequence
  Human MASP2 CCP1-CCP2-SP
MGSSHHHHHHSSGLVPRGSHMTGWKIHYTSTAQPCPYPMAPPNGHVSPVQAKYILKDSFSIFCETGYELLQGHLPLKSFTAVCQKDGSWDRPMPACSIVDCGPPDDLPSGRVEYITGPGVTTYKAVIQYSCEETFYTMKVNDGKYVCEADGFWTSSKGEKSLPVCEPVCGLSARTTGGRIYGGQKAKPGDFPWQVLILGGTTAAGALLYDNWVLTAAHAVYEQKHDASALDIRMGTLKRLSPHYTQAWSEAVFIHEGYTHDAGFDNDIALIKLNNKVVINSNITPICLPRKEAESFMRTDDIGTASGWGLTQRGFLARNLMYVDIPIVDHQKCTAAYEKPPYPRGSVTANMLCAGLESGGKDSCRGDAGGALVFLDSETERWFVGGIVSWGSMNCGEAGQYGVYTKVINYIPWIENIISDF

SEQ ID NO: 5 - protein, 345 aa, Artificial sequence
  Human MASP2 CCP2-SP
MGSSHHHHHHSSGLVPRGSHMIVDCGPPDDLPSGRVEYITGPGVTTYKAVIQYSCEETFYTMKVNDGKYVCEADGFWTSSKGEKSLPVCEPVCGLSARTTGGRIYGGQKAKPGDFPWQVLILGGTTAAGALLYDNWVLTAAHAVYEQKHDASALDIRMGTLKRLSPHYTQAWSEAVFIHEGYTHDAGFDNDIALIKLNNKVVINSNITPICLPRKEAESFMRTDDIGTASGWGLTQRGFLARNLMYVDIPIVDHQKCTAAYEKPPYPRGSVTANMLCAGLESGGKDSCRGDAGGALVFLDSETERWFVGGIVSWGSMNCGEAGQYGVYTKVINYIPWIENIISDF

SEQ ID NO: 6 - protein, 104 aa, Homo sapiens
MDAMKRGLCCVLLLCGAVFVSPSYTSTAHACPYPMAPPNGHVSPVQAKYILKDSFSIFCETGYELLQGHLPLKSFTAVCQKDGSWDRPMPACSAHHHHHHHHHH

SEQ ID NO: 7 - protein, 115 aa, Murine
DVQLQESGPGLVKPSQSLSLTCTVTGYSITSDYAWNWIRQFPGNKLEWMGYISYSGRTSYNPSLKSRISITRDTSKNQFFLQLNSVTTEDTATYYCAVLYALDYWGQGTSVTVSS

SEQ ID NO: 8 - protein, 107 aa, Murine
DIVMTQSQKFMSTSVGDRVSVTCKASQNVDTNVAWYQQKPGQSPKALIYSASYRYSGVPDRFTGSGSGTDFTLTISDVQSEDLAEYFCQQYNSNPLTFGSGTKLEIK

SEQ ID NO: 9 - protein, 115 aa, Murine
DVQLQESGPGLVKPSQSLSLTCTVTGYSITSDYAWNWIRQFPGNKLEWMGYISYSGRTSYNPSLKSRISITRDTSKNQFFLQLNSVTTEDTATYYCAILYAMNFWGQGTSVTVSS

SEQ ID NO: 10 - protein, 107 aa, Murine
DIVMTQSQKFMSTSVGDRVSVTCKASQNVDTNVAWYQQKPGQSPKALIYSASYRFSGVPDRFTGSGSGTDFTLTISNVQSEDLAEYFCQQYNSNPLTFGSGTKLEIK

SEQ ID NO: 11 - protein, 115 aa, Murine
DVQLQESGPGLVKPSQSLSLTCTVTGYSITSDYAWNWIRQFPGNKLEWMGYISYSGRTSYNPSLKSRISITRDTSKNQFFLQLNSVTTEDTATYYCAILYAMDYWGQGTSVTVSS

SEQ ID NO: 12 - protein, 107 aa, Murine
DIVMTQSQKFMSTSVGDRVSVTCKASQNVDTNVAWYQQKPGQSPKALIYSASYRYSGVPDRFTGSGSGTDFTLTISNVQSEDLAEYFCQQYNSNPLTFGSGTKLEIK

SEQ ID NO: 13 - protein, 122 aa, Murine
EVQLVESGGGLVKPGGSLKLSCAASGFTFSRFALSWVRQTPEKRLEWVAAVSRGGDYTYYPDSMKGRFTISRDNAMNTLYLQMSSLSSEDTAMYYCARHLYGYGHYYAMDYWGQGTSVTVSS

SEQ ID NO: 14 - protein, 107 aa, Murine
DIVMTQSHKFMSTSVGDRVSITCKASQDVNTAVAWYQQKPGQSPKLLIYSASYRYTGVPDRFTGSGSGTDFTFTISSVQAEDLAVYYCQQHYSTPYTFGGGTKLEIK

SEQ ID NO: 15 - protein, 122 aa, Murine
QVQLQESGPGLVKPSETLSLTCTVSGGSISSGEYFWGWIRQPPGKGLEWIGSIYYSGSTYYNPSLKSRVTISVDTSKNQFSLKLSSVTAADTAVYYCARSLKAARRDAFDIWGQGTTVTVSS

SEQ ID NO: 16 - protein, 106 aa, Murine
QSVLTQPPSVSVSPGQTASITCSGHKLGDKYAYWYQQKPGQSPVLVIYQDTKRPSGIPERFSGFNSGNTATLTISGTQATDEADYYCQTWDSSTGVFGAGTKVTVL

SEQ ID NO: 17 - protein, 6 aa, Murine
SDYAWN

SEQ ID NO: 18 - protein, 16 aa, Murine
YISYSGRTSYNPSLKS

SEQ ID NO: 19 - protein, 6 aa, Murine
LYALDY

SEQ ID NO: 20 - protein, 11 aa, Murine
KASQNVDTNVA

SEQ ID NO: 21 - protein, 7 aa, Murine
SASYRYS

SEQ ID NO: 22 - protein, 9 aa, Murine
QQYNSNPLT

SEQ ID NO: 23 - protein, 6 aa, Murine
LYAMNF

SEQ ID NO: 24 - protein, 7 aa, Murine
SASYRFS

SEQ ID NO: 25 - protein, 6 aa, Murine
LYAMDY

SEQ ID NO: 26 - protein, 6 aa, Artificial sequence
  HCDR3
  VARIANT (4)..(4): Xaa can be L or M
  VARIANT (5)..(5): Xaa can be D or N
  VARIANT (6)..(6): Xaa can be Y or F
LYAXXX

SEQ ID NO: 27 - protein, 7 aa, Artificial sequence
  LCDR2
  VARIANT (6)..(6): Xaa can be Y or F
SASYRXS

SEQ ID NO: 28 - protein, 5 aa, Murine
RFALS

SEQ ID NO: 29 - protein, 17 aa, Murine
AVSRGGDYTYYPDSMKG

SEQ ID NO: 30 - protein, 13 aa, Murine
HLYGYGHYYAMDY

SEQ ID NO: 31 - protein, 11 aa, Murine
KASQDVNTAVA

SEQ ID NO: 32 - protein, 7 aa, Murine
SASYRYT

SEQ ID NO: 33 - protein, 9 aa, Murine
QQHYSTPYT

SEQ ID NO: 34 - protein, 7 aa, Murine
SGEYFWG

SEQ ID NO: 35 - protein, 16 aa, Murine
SIYYSGSTYYNPSLKS

SEQ ID NO: 36 - protein, 12 aa, Murine
SLKAARRDAFDI

SEQ ID NO: 37 - protein, 11 aa, Murine
SGHKLGDKYAY

SEQ ID NO: 38 - protein, 7 aa, Murine
QDTKRPS

SEQ ID NO: 39 - protein, 9 aa, Murine
QTWDSSTGV

SEQ ID NO: 40 - protein, 445 aa, Artificial sequence
  Heavy chain of OMS721
QVTLKESGPVLVKPTETLTLTCTVSGFSLSRGKMGVSWIRQPPGKALEWLAHIFSSDEKSYRTSLKSRLTISKDTSKNQVVLTMTNMDPVDTATYYCARIRRGGIDYWGQGTLVTVSSASTKGPSVFPLAPCSRSTSESTAALGCLVKDYFPEPVTVSWNSGALTSGVHTFPAVLQSSGLYSLSSVVTVPSSSLGTKTYTCNVDHKPSNTKVDKRVESKYGPPCPPCPAPEFLGGPSVFLFPPKPKDTLMISRTPEVTCVVVDVSQEDPEVQFNWYVDGVEVHNAKTKPREEQFNSTYRVVSVLTVLHQDWLNGKEYKCKVSNKGLPSSIEKTISKAKGQPREPQVYTLPPSQEEMTKNQVSLTCLVKGFYPSDIAVEWESNGQPENNYKTTPPVLDSDGSFFLYSRLTVDKSRWQEGNVFSCSVMHEALHNHYTQKSLSLSLGK

SEQ ID NO: 41 - protein, 212 aa, Artificial sequence
  Light chain of OMS721
QPVLTQPPSLSVSPGQTASITCSGEKLGDKYAYWYQQKPGQSPVLVMYQDKQRPSGIPERFSGSNSGNTATLTISGTQAMDEADYYCQAWDSSTAVFGGGTKLTVLGQPKAAPSVTLFPPSSEELQANKATLVCLISDFYPGAVTVAWKADSSPVKAGVETTTPSKQSNNKYAASSYLSLTPEQWKSHRSYSCQVTHEGSTVEKTVAPTECS

SEQ ID NO: 42 - protein, 122 aa, Artificial sequence
  29C1 VH1
EVQLVESGGGLVKPGGSLRLSCAASGFTFSRFALSWVRQAPGKGLEWVSAVSRGGDYTYYPDSMKGRFTISRDNAKNSLYLQMNSLRAEDTAVYYCARHLYGYGHYYAMDYWGQGTTVTVSS

SEQ ID NO: 43 - protein, 122 aa, Artificial sequence
  29C1 VH2
EVQLVESGGGLVKPGGSLRLSCAASGFTFSRFALSWVRQAPGKGLEWVAAVSRGGDYTYYPDSMKGRFTISRDNAKNSLYLQMNSLRAEDTAVYYCARHLYGYGHYYAMDYWGQGTTVTVSS

SEQ ID NO: 44 - protein, 122 aa, Artificial sequence; identical to SEQ ID NO: 43
  29C1 VH3

SEQ ID NO: 45 - protein, 107 aa, Artificial sequence
  29C1 VL1
DIQMTQSPSSLSASVGDRVTITCKASQDVNTAVAWYQQKPGKAPKLLIYSASYRYTGVPSRFSGSGSGTDFTFTISSLQPEDIATYYCQQHYSTPYTFGGGTKVEIK

SEQ ID NO: 46 - protein, 107 aa, Artificial sequence
  29C1 VL2
DIVMTQSPSSLSASVGDRVTITCKASQDVNTAVAWYQQKPGKSPKLLIYSASYRYTGVPSRFSGSGSGTDFTFTISSLQPEDIATYYCQQHYSTPYTFGGGTKVEIK

SEQ ID NO: 47 - protein, 115 aa, Artificial sequence
  77H11 VH1
EVQLQESGPGLVKPSQTLSLTCTVSGGSISSDYAWNWIRQPPGKGLEWIGYISYSGRTSYNPSLKSRVTISVDTSKNQFSLKLSSVTAADTAVYYCAVLYALDYWGQGTTVTVSS

SEQ ID NO: 48 - protein, 115 aa, Artificial sequence
  77H11 VH2
EVQLQESGPGLVKPSQTLSLTCTVSGYSITSDYAWNWIRQPPGKGLEWIGYISYSGRTSYNPSLKSRVTISVDTSKNQFSLKLSSVTAADTAVYYCAVLYALDYWGQGTTVTVSS

SEQ ID NO: 49 - protein, 115 aa, Artificial sequence
  77H11 VH3
EVQLQESGPGLVKPSQTLSLTCTVSGYSITSDYAWNWIRQPPGKGLEWIGYISYSGRTSYNPSLKSRVTISRDTSKNQFSLKLSSVTAADTAVYYCAVLYALDYWGQGTTVTVSS

SEQ ID NO: 50 - protein, 115 aa, Artificial sequence
  77H11 VH4
EVQLQESGPGLVKPSQTLSLTCTVSGYSITSDYAWNWIRQPPGNKLEWMGYISYSGRTSYNPSLKSRITISRDTSKNQFSLKLSSVTAADTAVYYCAVLYALDYWGQGTTVTVSS

SEQ ID NO: 51 - protein, 107 aa, Artificial sequence
  77H11 VL1
DIQMTQSPSSLSASVGDRVTITCKASQNVDTNVAWYQQKPGKVPKALIYSASYRYSGVPSRFSGSGSGTDFTLTISSLQPEDVATYYCQQYNSNPLTFGQGTKLEIK

SEQ ID NO: 52 - protein, 107 aa, Artificial sequence
  77H11 VL2
DIQMTQSPSSLSASVGDRVTITCKASQNVDTNVAWYQQKPGKSPKALIYSASYRYSGVPSRFSGSGSGTDFTLTISSLQPEDVAEYYCQQYNSNPLTFGQGTKLEIK

SEQ ID NO: 53 - protein, 327 aa, Artificial sequence
  Human IgG4 Fc
ASTKGPSVFPLAPCSRSTSESTAALGCLVKDYFPEPVTVSWNSGALTSGVHTFPAVLQSSGLYSLSSVVTVPSSSLGTKTYTCNVDHKPSNTKVDKRVESKYGPPCPPCPAPEFLGGPSVFLFPPKPKDTLMISRTPEVTCVVVDVSQEDPEVQFNWYVDGVEVHNAKTKPREEQFNSTYRVVSVLTVLHQDWLNGKEYKCKVSNKGLPSSIEKTISKAKGQPREPQVYTLPPSQEEMTKNQVSLTCLVKGFYPSDIAVEWESNGQPENNYKTTPPVLDSDGSFFLYSRLTVDKSRWQEGNVFSCSVMHEALHNHYTQKSLSLSLGK

SEQ ID NO: 54 - protein, 449 aa, Artificial sequence
  Heavy chain of 29C1
EVQLVESGGGLVKPGGSLRLSCAASGFTFSRFALSWVRQAPGKGLEWVSAVSRGGDYTYYPDSMKGRFTISRDNAKNSLYLQMNSLRAEDTAVYYCARHLYGYGHYYAMDYWGQGTTVTVSSASTKGPSVFPLAPCSRSTSESTAALGCLVKDYFPEPVTVSWNSGALTSGVHTFPAVLQSSGLYSLSSVVTVPSSSLGTKTYTCNVDHKPSNTKVDKRVESKYGPPCPPCPAPEFLGGPSVFLFPPKPKDTLMISRTPEVTCVVVDVSQEDPEVQFNWYVDGVEVHNAKTKPREEQFNSTYRVVSVLTVLHQDWLNGKEYKCKVSNKGLPSSIEKTISKAKGQPREPQVYTLPPSQEEMTKNQVSLTCLVKGFYPSDIAVEWESNGQPENNYKTTPPVLDSDGSFFLYSRLTVDKSRWQEGNVFSCSVMHEALHNHYTQKSLSLSLGK

SEQ ID NO: 55 - protein, 214 aa, Artificial sequence
  Light chain of 29C1
DIQMTQSPSSLSASVGDRVTITCKASQDVNTAVAWYQQKPGKAPKLLIYSASYRYTGVPSRFSGSGSGTDFTFTISSLQPEDIATYYCQQHYSTPYTFGGGTKVEIKRTVAAPSVFIFPPSDEQLKSGTASVVCLLNNFYPREAKVQWKVDNALQSGNSQESVTEQDSKDSTYSLSSTLTLSKADYEKHKVYACEVTHQGLSSPVTKSFNRGEC

SEQ ID NO: 56 - protein, 442 aa, Artificial sequence
  Heavy chain of 77H11
EVQLQESGPGLVKPSQTLSLTCTVSGYSITSDYAWNWIRQPPGKGLEWIGYISYSGRTSYNPSLKSRVTISRDTSKNQFSLKLSSVTAADTAVYYCAVLYALDYWGQGTTVTVSSASTKGPSVFPLAPCSRSTSESTAALGCLVKDYFPEPVTVSWNSGALTSGVHTFPAVLQSSGLYSLSSVVTVPSSSLGTKTYTCNVDHKPSNTKVDKRVESKYGPPCPPCPAPEFLGGPSVFLFPPKPKDTLMISRTPEVTCVVVDVSQEDPEVQFNWYVDGVEVHNAKTKPREEQFNSTYRVVSVLTVLHQDWLNGKEYKCKVSNKGLPSSIEKTISKAKGQPREPQVYTLPPSQEEMTKNQVSLTCLVKGFYPSDIAVEWESNGQPENNYKTTPPVLDSDGSFFLYSRLTVDKSRWQEGNVFSCSVMHEALHNHYTQKSLSLSLGK

SEQ ID NO: 57 - protein, 214 aa, Artificial sequence
  Light chain of 77H11
DIQMTQSPSSLSASVGDRVTITCKASQNVDTNVAWYQQKPGKVPKALIYSASYRYSGVPSRFSGSGSGTDFTLTISSLQPEDVATYYCQQYNSNPLTFGQGTKLEIKRTVAAPSVFIFPPSDEQLKSGTASVVCLLNNFYPREAKVQWKVDNALQSGNSQESVTEQDSKDSTYSLSSTLTLSKADYEKHKVYACEVTHQGLSSPVTKSFNRGEC

SEQ ID NO: 58 - protein, 449 aa, Artificial sequence
  Heavy chain of 11165
QVQLQESGPGLVKPSETLSLTCTVSGGSISSGEYFWGWIRQPPGKGLEWIGSIYYSGSTYYNPSLKSRVTISVDTSKNQFSLKLSSVTAADTAVYYCARSLKAARRDAFDIWGQGTTVTVSSASTKGPSVFPLAPCSRSTSESTAALGCLVKDYFPEPVTVSWNSGALTSGVHTFPAVLQSSGLYSLSSVVTVPSSSLGTKTYTCNVDHKPSNTKVDKRVESKYGPPCPPCPAPEFLGGPSVFLFPPKPKDTLMISRTPEVTCVVVDVSQEDPEVQFNWYVDGVEVHNAKTKPREEQFNSTYRVVSVLTVLHQDWLNGKEYKCKVSNKGLPSSIEKTISKAKGQPREPQVYTLPPSQEEMTKNQVSLTCLVKGFYPSDIAVEWESNGQPENNYKTTPPVLDSDGSFFLYSRLTVDKSRWQEGNVFSCSVMHEALHNHYTQKSLSLSLGK

SEQ ID NO: 59 - protein, 212 aa, Artificial sequence
  Light chain of 11165
QSVLTQPPSVSVSPGQTASITCSGHKLGDKYAYWYQQKPGQSPVLVIYQDTKRPSGIPERFSGFNSGNTATLTISGTQATDEADYYCQTWDSSTGVFGAGTKVTVLGQPKANPTVTLFPPSSEELQANKATLVCLISDFYPGAVTVAWKADGSPVKAGVETTKPSKQSNNKYAASSYLSLTPEQWKSHRSYSCQVTHEGSTVEKTVAPTECS

SEQ ID NO: 60 - protein, 15 aa, Artificial sequence
  Signal peptide
MRLLTLLGLLCGSVA

SEQ ID NO: 61 - protein, 19 aa, Artificial sequence
  Signal peptide
MEFGLSWLFLVAILKGVQC